European Patent Specification EP 3 872 177 B1, published November 26, 2025. Title: COMPOSITIONS AND METHODS FOR ENHANCING HOMOLOGOUS RECOMBINATION. Applicant: LIFE TECHNOLOGIES CORPORATION. Application PCT/US2017/034520. The sequence listing filed with the application follows.

SEQUENCE LISTING (127 sequences)

SEQ ID NO: 1 - RNA, 104 nt, Artificial Sequence
  source: /note="Description of Artificial Sequence: Synthetic polynucleotide"
gcauuucgguaugcauaugaaugaguuuuagagcuagaaauagcaaguuaaaauaaggcuaguccguuaucaacuugaaaaaguggcaccgagucggugcuuuu

SEQ ID NO: 2 - DNA, 23 bp, Artificial Sequence
  source: /note="Description of Artificial Sequence: Synthetic oligonucleotide"
cgtaaagccatacgtatactacc

SEQ ID NO: 3 - DNA, 23 bp, Artificial Sequence
  source: /note="Description of Artificial Sequence: Synthetic oligonucleotide"
  modified_base (21)..(21): a, c, t, g, unknown or other
gcatttcggtatgcatatgangg

SEQ ID NO: 4 - DNA, 48 bp, Artificial Sequence
  source: /note="Description of Artificial Sequence: Synthetic oligonucleotide"
tcgtgaccaccctgacccacggcgtgcagtgcttcagccgctaccccg

SEQ ID NO: 5 - DNA, 48 bp, Artificial Sequence
  source: /note="Description of Artificial Sequence: Synthetic oligonucleotide"
tcgtgaccaccctgacctacggcgtgcagtgcttcagccgctaccccg

SEQ ID NO: 6 - DNA, 66 bp, Artificial Sequence
  source: /note="Description of Artificial Sequence: Synthetic oligonucleotide"
tcgtgaccaccctgacctacggcgtgcagtgcttcagcggcgtgcagtgcttcagccgctaccccg

SEQ ID NO: 7 - DNA, 38 bp, Artificial Sequence
  source: /note="Description of Artificial Sequence: Synthetic oligonucleotide"
tcgtgactacggcgtgcagtgcttcagccgctaccccg

SEQ ID NO: 8 - DNA, 47 bp, Artificial Sequence
  source: /note="Description of Artificial Sequence: Synthetic oligonucleotide"
tcgtgaccaccctgaccacggcgtgcagtgcttcagccgctaccccg

SEQ ID NO: 9 - DNA, 38 bp, Artificial Sequence
  source: /note="Description of Artificial Sequence: Synthetic oligonucleotide"
tcgaggccacggcgtgcagtgcttcagccgctaccccg

SEQ ID NO: 10 - DNA, 33 bp, Artificial Sequence
  source: /note="Description of Artificial Sequence: Synthetic oligonucleotide"
tctacggcgtgcagtgcttcagccgctaccccg

SEQ ID NO: 11 - DNA, 32 bp, Artificial Sequence
  source: /note="Description of Artificial Sequence: Synthetic oligonucleotide"
tcgtggcgtgcagtgcttcagccgctaccccg

SEQ ID NO: 12 - DNA, 31 bp, Artificial Sequence
  source: /note="Description of Artificial Sequence: Synthetic oligonucleotide"
tcgtgcgtgcagtgcttcagccgctaccccg

SEQ ID NO: 13 - DNA, 22 bp, Artificial Sequence
  source: /note="Description of Artificial Sequence: Synthetic oligonucleotide"
tcgtgaccaagccgctaccccg

SEQ ID NO: 14 - DNA, 14 bp, Artificial Sequence
  source: /note="Description of Artificial Sequence: Synthetic oligonucleotide"
tcgtgaccaccccg

SEQ ID NO: 15 - DNA, 20 bp, Artificial Sequence
  source: /note="Description of Artificial Sequence: Synthetic oligonucleotide"
gaccaccctgacccacggcg

SEQ ID NO: 16 - DNA, 50 bp, Artificial Sequence
  source: /note="Description of Artificial Sequence: Synthetic oligonucleotide"
gaccaccctgaccgactacaaagacgatgacgacaagaattcttacggcg

SEQ ID NO: 17 - DNA, 50 bp, Artificial Sequence
  source: /note="Description of Artificial Sequence: Synthetic oligonucleotide"
gaccaccctgcccgactacaaagacgatgacgacaagaattcttacggcg

SEQ ID NO: 18 - DNA, 49 bp, Artificial Sequence
  source: /note="Description of Artificial Sequence: Synthetic oligonucleotide"
gaccaccctgccgactacaaagacgatgacgacaagaattcttacggcg

SEQ ID NO: 19 - DNA, 73 bp, Artificial Sequence
  source: /note="Description of Artificial Sequence: Synthetic oligonucleotide"
gaccaccctggcctgcaccctcgtgacaccctgaccgactacaaagacgatgacgacaagtattcttacggcg

SEQ ID NO: 20 - DNA, 44 bp, Artificial Sequence
  source: /note="Description of Artificial Sequence: Synthetic oligonucleotide"
gaccaccctgaccgactacaaagacgacaagaattcttacggcg

SEQ ID NO: 21 - DNA, 35 bp, Artificial Sequence
  source: /note="Description of Artificial Sequence: Synthetic oligonucleotide"
gaccgactacaaagacgacaagaattcttacggcg

SEQ ID NO: 22 - DNA, 31 bp, Artificial Sequence
  source: /note="Description of Artificial Sequence: Synthetic oligonucleotide"
gaccgacgatgacgacaaaattcttacggcg

SEQ ID NO: 23 - DNA, 10 bp, Artificial Sequence
  source: /note="Description of Artificial Sequence: Synthetic oligonucleotide"
gaccacggcg

SEQ ID NO: 24 - DNA, 12 bp, Artificial Sequence
  source: /note="Description of Artificial Sequence: Synthetic oligonucleotide"
gaccccacggcg

SEQ ID NO: 25 - DNA, 6 bp, Artificial Sequence
  source: /note="Description of Artificial Sequence: Synthetic oligonucleotide"
cacctt

SEQ ID NO: 26 - protein, 7 aa, Artificial Sequence
  source: /note="Description of Artificial Sequence: Synthetic peptide"
VTTFTYG

SEQ ID NO: 27 - DNA, 21 bp, Artificial Sequence
  source: /note="Description of Artificial Sequence: Synthetic oligonucleotide"
  CDS (1)..(21)
gtgaccaccttcacctacggc

SEQ ID NO: 28 - protein, 5 aa, Artificial Sequence
  source: /note="Description of Artificial Sequence: Synthetic peptide"
VTTYG

SEQ ID NO: 29 - DNA, 15 bp, Artificial Sequence
  source: /note="Description of Artificial Sequence: Synthetic oligonucleotide"
  CDS (1)..(15)
gtgaccacctacggc

SEQ ID NO: 30 - protein, 4 aa, Artificial Sequence
  source: /note="Description of Artificial Sequence: Synthetic peptide"
LTHG

SEQ ID NO: 31 - DNA, 12 bp, Artificial Sequence
  source: /note="Description of Artificial Sequence: Synthetic oligonucleotide"
  CDS (1)..(12)
ctgacccacggc

SEQ ID NO: 32 - protein, 4 aa, Artificial Sequence
  source: /note="Description of Artificial Sequence: Synthetic peptide"
LTYG

SEQ ID NO: 33 - DNA, 12 bp, Artificial Sequence
  source: /note="Description of Artificial Sequence: Synthetic oligonucleotide"
  CDS (1)..(12)
ctgacctacggc

SEQ ID NO: 34 - protein, 887 aa, Natronobacterium gregoryi
MTVIDLDSTTTADELTSGHTYDISVTLTGVYDNTDEQHPRMSLAFEQDNGERRYITLWKNTTPKDVFTYDYATGSTYIFTNIDYEVKDGYENLTATYQTTVENATAQEVGTTDEDETFAGGEPLDHHLDDALNETPDDAETESDSGHVMTSFASRDQLPEWTLHTYTLTATDGAKTDTEYARRTLAYTVRQELYTDHDAAPVATDGLMLLTPEPLGETPLDLDCGVRVEADETRTLDYTTAKDRLLARELVEEGLKRSLWDDYLVRGIDEVLSKEPVLTCDEFDLHERYDLSVEVGHSGRAYLHINFRHRFVPKLTLADIDDDNIYPGLRVKTTYRPRRGHIVWGLRDECATDSLNTLGNQSVVAYHRNNQTPINTDLLDAIEAADRRVVETRRQGHGDDAVSFPQELLAVEPNTHQIKQFASDGFHQQARSKTRLSASRCSEKAQAFAERLDPVRLNGSTVEFSSEFFTGNNEQQLRLLYENGESVLTFRDGARGAHPDETFSKGIVNPPESFEVAVVLPEQQADTCKAQWDTMADLLNQAGAPPTRSETVQYDAFSSPESISLNVAGAIDPSEVDAAFVVLPPDQEGFADLASPTETYDELKKALANMGIYSQMAYFDRFRDAKIFYTRNVALGLLAAAGGVAFTTEHAMPGDADMFIGIDVSRSYPEDGASGQINIAATATAVYKDGTILGHSSTRPQLGEKLQSTDVRDIMKNAILGYQQVTGESPTHIVIHRDGFMNEDLDPATEFLNEQGVEYDIVEIRKQPQTRLLAVSDVQYDTPVKSIAAINQNEPRATVATFGAPEYLATRDGGGLPRPIQIERVAGETDIETLTRQVYLLSQSHIQVHNSTARLPITTAYADQASTHATKGYLVQTGAFESNVGFL

SEQ ID NO: 35 - DNA, 97 bp, Artificial Sequence
  source: /note="Description of Artificial Sequence: Synthetic oligonucleotide"
catctgcaccaccggcaagctgcccgtgccctggcccaccctcgtgaccaccttcacctacggcgtgcagtgcttcgcccgctaccccgaccacatg

SEQ ID NO: 36 - DNA, 97 bp, Artificial Sequence
  source: /note="Description of Artificial Sequence: Synthetic oligonucleotide"
catgtggtcggggtagcgggcgaagcactgcacgccgtaggtgaaggtggtcacgagggtgggccagggcacgggcagcttgccggtggtgcagatg

SEQ ID NO: 37 - DNA, 97 bp, Artificial Sequence; identical to SEQ ID NO: 36
  source: /note="Description of Artificial Sequence: Synthetic oligonucleotide"

SEQ ID NO: 38 - DNA, 79 bp, Artificial Sequence
  source: /note="Description of Artificial Sequence: Synthetic oligonucleotide"
catgtggtcggggtagcgggcgaagcactgcacgccgtaggtgaaggtggtcacgagggtgggccagggcacgggcagc

SEQ ID NO: 39 - DNA, 79 bp, Artificial Sequence; identical to SEQ ID NO: 38
  source: /note="Description of Artificial Sequence: Synthetic oligonucleotide"

SEQ ID NO: 40 - DNA, 60 bp, Artificial Sequence
  source: /note="Description of Artificial Sequence: Synthetic oligonucleotide"
cggggtagcgggcgaagcactgcacgccgtaggtgaaggtggtcacgagggtgggccagg

SEQ ID NO: 41 - DNA, 60 bp, Artificial Sequence; identical to SEQ ID NO: 40
  source: /note="Description of Artificial Sequence: Synthetic oligonucleotide"

SEQ ID NO: 42 - DNA, 40 bp, Artificial Sequence
  source: /note="Description of Artificial Sequence: Synthetic oligonucleotide"
ggcgaagcactgcacgccgtaggtgaaggtggtcacgagg

SEQ ID NO: 43 - DNA, 40 bp, Artificial Sequence; identical to SEQ ID NO: 42
  source: /note="Description of Artificial Sequence: Synthetic oligonucleotide"

SEQ ID NO: 44 - DNA, 100 bp, Artificial Sequence
  source: /note="Description of Artificial Sequence: Synthetic polynucleotide"
accggcaagctgcccgtgccctggcccaccctcgtgaccaccctgacctacggcgtgcagtgcttcagccgctaccccgaccacatgaagcagcacgact

SEQ ID NO: 45 - DNA, 99 bp, Artificial Sequence
  source: /note="Description of Artificial Sequence: Synthetic oligonucleotide"
accggcaagctgcccgtgccctggcccaccctctgaccaccctgacctacggcgtgcagtgcttcagccgctaccccgaccacatgaagcagcacgact

SEQ ID NO: 46 - DNA, 90 bp, Artificial Sequence
  source: /note="Description of Artificial Sequence: Synthetic oligonucleotide"
gcaagctgcccgtgccctggcccaccctcgtgaccaccctgacctacggcgtgcagtgcttcagccgctaccccgaccacatgaagcagc

SEQ ID NO: 47 - DNA, 90 bp, Artificial Sequence; identical to SEQ ID NO: 46
  source: /note="Description of Artificial Sequence: Synthetic oligonucleotide"

SEQ ID NO: 48 - DNA, 80 bp, Artificial Sequence
  source: /note="Description of Artificial Sequence: Synthetic oligonucleotide"
gctgcccgtgccctggcccaccctcgtgaccaccctgacctacggcgtgcagtgcttcagccgctaccccgaccacatga

SEQ ID NO: 49 - DNA, 80 bp, Artificial Sequence; identical to SEQ ID NO: 48
  source: /note="Description of Artificial Sequence: Synthetic oligonucleotide"

SEQ ID NO: 50 - DNA, 70 bp, Artificial Sequence
  source: /note="Description of Artificial Sequence: Synthetic oligonucleotide"
cccgtgccctggcccaccctcgtgaccaccctgacctacggcgtgcagtgcttcagccgctaccccgacc

SEQ ID NO: 51 - DNA, 70 bp, Artificial Sequence; identical to SEQ ID NO: 50
  source: /note="Description of Artificial Sequence: Synthetic oligonucleotide"

SEQ ID NO: 52 - DNA, 60 bp, Artificial Sequence
  source: /note="Description of Artificial Sequence: Synthetic oligonucleotide"
gccctggcccaccctcgtgaccaccctgacctacggcgtgcagtgcttcagccgctaccc

SEQ ID NO: 53 - DNA, 60 bp, Artificial Sequence; identical to SEQ ID NO: 52
  source: /note="Description of Artificial Sequence: Synthetic oligonucleotide"

SEQ ID NO: 54 - DNA, 50 bp, Artificial Sequence
  source: /note="Description of Artificial Sequence: Synthetic oligonucleotide"
cccaccctcgtgaccaccctgacctacggcgtgcagtgcttcagccgcta

SEQ ID NO: 55 - DNA, 50 bp, Artificial Sequence; identical to SEQ ID NO: 54
  source: /note="Description of Artificial Sequence: Synthetic oligonucleotide"

SEQ ID NO: 56 - DNA, 80 bp, Artificial Sequence
  source: /note="Description of Artificial Sequence: Synthetic oligonucleotide"
gcgtatcaatggatacttacattgactaatccaaactagtgctcattgaccggaaactgttctggaccaatctctttctc

SEQ ID NO: 57 - DNA, 83 bp, Artificial Sequence
  source: /note="Description of Artificial Sequence: Synthetic oligonucleotide"
gcaatccagtgaatccttgaggtgtaacgtggagccagtaaggcggctacatatctttagtggtgcccatggaccagaaaaag

SEQ ID NO: 58 - DNA, 81 bp, Artificial Sequence
  source: /note="Description of Artificial Sequence: Synthetic oligonucleotide"
ctgcacggggctgctggcgctcacatttcctattcctggattgatactagagccgctgcctcctcgtagaagctccgacag

SEQ ID NO: 59 - DNA, 98 bp, Artificial Sequence
  source: /note="Description of Artificial Sequence: Synthetic oligonucleotide"
ctgaccttgccttcatgtgattcagccccagtccattaccctgtgtaggactgagaaatgcaagactctggctagagttccttcttccatctcccttc

SEQ ID NO: 60 - DNA, 98 bp, Artificial Sequence
  source: /note="Description of Artificial Sequence: Synthetic oligonucleotide"
ctgaccttgccttcatgtgattcagccccagtccattacactgtgtaggactgagaaatgcaagactctggctagagttccttcttccatctcccttc

SEQ ID NO: 61 - DNA, 97 bp, Artificial Sequence
  source: /note="Description of Artificial Sequence: Synthetic oligonucleotide"
ctgaagttcatctgcaccaccggcaagctgcccgtgccctggcccaccctcgtgaccaccttcacctacggcgtgcagtgcttcgcccgctaccccg

SEQ ID NO: 62 - DNA, 97 bp, Artificial Sequence
  source: /note="Description of Artificial Sequence: Synthetic oligonucleotide"
cggggtagcgggcgaagcactgcacgccgtaggtgaaggtggtcacgagggtgggccagggcacgggcagcttgccggtggtgcagatgaacttcag

SEQ ID NO: 63 - DNA, 97 bp, Artificial Sequence
  source: /note="Description of Artificial Sequence: Synthetic oligonucleotide"
ccgtgccctggcccaccctcgtgaccaccttcacctacggcgtgcagtgcttcgcccgctaccccgaccacatgaagcagcacgacttcttcaagtc

SEQ ID NO: 64 - DNA, 97 bp, Artificial Sequence
  source: /note="Description of Artificial Sequence: Synthetic oligonucleotide"
gacttgaagaagtcgtgctgcttcatgtggtcggggtagcgggcgaagcactgcacgccgtaggtgaaggtggtcacgagggtgggccagggcacgg

SEQ ID NO: 65 - DNA, 81 bp, Artificial Sequence
  source: /note="Description of Artificial Sequence: Synthetic oligonucleotide"
ccaccggcaagctgcccgtgccctggcccaccctcgtgaccaccttcacctacggcgtgcagtgcttcgcccgctaccccg

SEQ ID NO: 66 - DNA, 81 bp, Artificial Sequence
  source: /note="Description of Artificial Sequence: Synthetic oligonucleotide"
cggggtagcgggcgaagcactgcacgccgtaggtgaaggtggtcacgagggtgggccagggcacgggcagcttgccggtgg

SEQ ID NO: 67 - DNA, 81 bp, Artificial Sequence
  source: /note="Description of Artificial Sequence: Synthetic oligonucleotide"
ccgtgccctggcccaccctcgtgaccaccttcacctacggcgtgcagtgcttcgcccgctaccccgaccacatgaagcagc

SEQ ID NO: 68 - DNA, 81 bp, Artificial Sequence
  source: /note="Description of Artificial Sequence: Synthetic oligonucleotide"
gctgcttcatgtggtcggggtagcgggcgaagcactgcacgccgtaggtgaaggtggtcacgagggtgggccagggcacgg

SEQ ID NO: 69 - DNA, 98 bp, Artificial Sequence
  source: /note="Description of Artificial Sequence: Synthetic oligonucleotide"
ccaccggcaagctgcccgtgccctggcccaccctcgtgaccaccttcacctacggcgtgcagtgcttcgcccgctaccccgaccacatgaagcagcac

SEQ ID NO: 70 - DNA, 97 bp, Artificial Sequence
  source: /note="Description of Artificial Sequence: Synthetic oligonucleotide"
gtgctgcttcatgtggtcggggtagcgggcgaagcactgcacgccgtaggtgaaggtggcacgagggtgggccagggcacgggcagcttgccggtgg

SEQ ID NO: 71 - DNA, 82 bp, Artificial Sequence
  source: /note="Description of Artificial Sequence: Synthetic oligonucleotide"
caagctgcccgtgccctggcccaccctcgtgaccaccttcacctacggcgtgcagtgcttcgcccgctaccccgaccacatg

SEQ ID NO: 72 - DNA, 82 bp, Artificial Sequence
  source: /note="Description of Artificial Sequence: Synthetic oligonucleotide"
catgtggtcggggtagcgggcgaagcactgcacgccgtaggtgaaggtggtcacgagggtgggccagggcacgggcagcttg

SEQ ID NO: 73 - skipped

SEQ ID NO: 74 - DNA, 99 bp, Artificial Sequence
  source: /note="Description of Artificial Sequence: Synthetic oligonucleotide"
gtgccctggcccaccctcgtgaccaccctgaccgactacaaagacgatgacgacaagaattcttacggcgtgcagtgcttcagccgctaccccgaccac

SEQ ID NO: 75 - DNA, 31 bp, Artificial Sequence
  source: /note="Description of Artificial Sequence: Synthetic oligonucleotide"
gactacaaagacgatgacgacaagaattctt

SEQ ID NO: 76 - DNA, 31 bp, Artificial Sequence
  source: /note="Description of Artificial Sequence: Synthetic oligonucleotide"
aagaattcttgtcgtcatcgtctttgtagtc

SEQ ID NO: 77 - DNA, 37 bp, Artificial Sequence
  source: /note="Description of Artificial Sequence: Synthetic oligonucleotide"
ctgaccgactacaaagacgatgacgacaagaattctt

SEQ ID NO: 78 - DNA, 37 bp, Artificial Sequence
  source: /note="Description of Artificial Sequence: Synthetic oligonucleotide"
cgccgtaagaattcttgtcgtcatcgtctttgtagtc

SEQ ID NO: 79 - DNA, 37 bp, Artificial Sequence
  source: /note="Description of Artificial Sequence: Synthetic oligonucleotide"
gactacaaagacgatgacgacaagaattcttacggcg

SEQ ID NO: 80 - DNA, 37 bp, Artificial Sequence
  source: /note="Description of Artificial Sequence: Synthetic oligonucleotide"
aagaattcttgtcgtcatcgtctttgtagtcggtcag

SEQ ID NO: 81 - DNA, 46 bp, Artificial Sequence
  source: /note="Description of Artificial Sequence: Synthetic oligonucleotide"
gtgaccaccctgaccgactacaaagacgatgacgacaagaattctt

SEQ ID NO: 82 - DNA, 45 bp, Artificial Sequence
  source: /note="Description of Artificial Sequence: Synthetic oligonucleotide"
gcactgcacgccgtaagaattcttgtcgtcatcgtctttgtagtc

SEQ ID NO: 83 - DNA, 45 bp, Artificial Sequence
  source: /note="Description of Artificial Sequence: Synthetic oligonucleotide"
gactacaaagacgatgacgacaagaattcttacggcgtgcagtgc

SEQ ID NO: 84 - DNA, 46 bp, Artificial Sequence
  source: /note="Description of Artificial Sequence: Synthetic oligonucleotide"
aagaattcttgtcgtcatcgtctttgtagtcggtcagggtggtcac

SEQ ID NO: 85 - DNA, 64 bp, Artificial Sequence
  source: /note="Description of Artificial Sequence: Synthetic oligonucleotide"
gtgccctggcccaccctcgtgaccaccctgaccgactacaaagacgatgacgacaagaattctt

SEQ ID NO: 86 - DNA, 66 bp, Artificial Sequence
  source: /note="Description of Artificial Sequence: Synthetic oligonucleotide"
gtggtcggggtagcggctgaagcactgcacgccgtaagaattcttgtcgtcatcgtctttgtagtc

SEQ ID NO: 87 - DNA, 66 bp, Artificial Sequence
  source: /note="Description of Artificial Sequence: Synthetic oligonucleotide"
gactacaaagacgatgacgacaagaattcttacggcgtgcagtgcttcagccgctaccccgaccac

SEQ ID NO: 88 - DNA, 64 bp, Artificial Sequence
  source: /note="Description of Artificial Sequence: Synthetic oligonucleotide"
aagaattcttgtcgtcatcgtctttgtagtcggtcagggtggtcacgagggtgggccagggcac

SEQ ID NO: 89 - DNA, 60 bp, Artificial Sequence
  source: /note="Description of Artificial Sequence: Synthetic oligonucleotide"
gactacaaagacgatgacgacaagaattcttacggcgtgcagtgcttcagccgctacccc

SEQ ID NO: 90 - DNA, 58 bp, Artificial Sequence
  source: /note="Description of Artificial Sequence: Synthetic oligonucleotide"
aagaattcttgtcgtcatcgtctttgtagtcggtcagggtggtcacgagggtgggcca

SEQ ID NO: 91 - DNA, 66 bp, Artificial Sequence; identical to SEQ ID NO: 87
  source: /note="Description of Artificial Sequence: Synthetic oligonucleotide"

SEQ ID NO: 92 - DNA, 64 bp, Artificial Sequence; identical to SEQ ID NO: 88
  source: /note="Description of Artificial Sequence: Synthetic oligonucleotide"

SEQ ID NO: 93 - DNA, 67 bp, Artificial Sequence
  source: /note="Description of Artificial Sequence: Synthetic oligonucleotide"
aagaattcttgtcgtcatcgtctttgtagtcggtcagggtggtcacgagggtgggccagggcacggg

SEQ ID NO: 94 - DNA, 66 bp, Artificial Sequence; identical to SEQ ID NO: 87
  source: /note="Description of Artificial Sequence: Synthetic oligonucleotide"

SEQ ID NO: 95 - DNA, 78 bp, Artificial Sequence
  source: /note="Description of Artificial Sequence: Synthetic oligonucleotide"
gactacaaagacgatgacgacaagaattcttacggcgtgcagtgcttcagccgctaccccgaccacatgaagcagcac

SEQ ID NO: 96 - DNA, 78 bp, Artificial Sequence
  source: /note="Description of Artificial Sequence: Synthetic oligonucleotide"
aagaattcttgtcgtcatcgtctttgtagtcggtcagggtggtcacgagggtgggccagggcacgggcagcttgccgg

SEQ ID NO: 97 - DNA, 94 bp, Artificial Sequence
  source: /note="Description of Artificial Sequence: Synthetic oligonucleotide"
gcccgtgccctggcccaccctcgtgaccacctgactacaaagacgatgacgacaagaattctacggcgtgcagtgcttcgcccgctaccccgac

SEQ ID NO: 98 - DNA, 63 bp, Artificial Sequence
  source: /note="Description of Artificial Sequence: Synthetic oligonucleotide"
gcccgtgccctggcccaccctcgtgaccacctgactacaaagacgatgacgacaagaattcta

SEQ ID NO: 99 - DNA, 62 bp, Artificial Sequence
  source: /note="Description of Artificial Sequence: Synthetic oligonucleotide"
gtcggggtagcgggcgaagcactgcacgccgtagaattcttgtcgtcatcgtctttgtagtc

SEQ ID NO: 100 - DNA, 62 bp, Artificial Sequence
  source: /note="Description of Artificial Sequence: Synthetic oligonucleotide"
agaattcttgtcgtcatcgtctttgtagtcaggtggtcacgagggtgggccagggcacgggc

SEQ ID NO: 101 - DNA, 62 bp, Artificial Sequence
  source: /note="Description of Artificial Sequence: Synthetic oligonucleotide"
gactacaaagacgatgacgacaagaattctacggcgtgcagtgcttcgcccgctaccccgac

SEQ ID NO: 102 - DNA, 23 bp, Artificial Sequence
  source: /note="Description of Artificial Sequence: Synthetic primer"
ctcgtgaccaccctgacccacgg

SEQ ID NO: 103 - DNA, 23 bp, Artificial Sequence
  source: /note="Description of Artificial Sequence: Synthetic primer"
ctgaagttcatctgcaccaccgg

SEQ ID NO: 104 - DNA, 23 bp, Artificial Sequence
  source: /note="Description of Artificial Sequence: Synthetic primer"
gggcacgggcagcttgccggtgg

SEQ ID NO: 105 - DNA, 23 bp, Artificial Sequence
  source: /note="Description of Artificial Sequence: Synthetic primer"
ccagggcacgggcagcttgccgg

SEQ ID NO: 106 - DNA, 21 bp, Artificial Sequence
  source: /note="Description of Artificial Sequence: Synthetic primer"
ggcaagctgcccgtgccctgg

SEQ ID NO: 107 - DNA, 23 bp, Artificial Sequence
  source: /note="Description of Artificial Sequence: Synthetic primer"
cacgagggtgggccagggcacgg

SEQ ID NO: 108 - DNA, 23 bp, Artificial Sequence
  source: /note="Description of Artificial Sequence: Synthetic primer"
ggtggtcacgagggtgggccagg

SEQ ID NO: 109 - DNA, 23 bp, Artificial Sequence
  source: /note="Description of Artificial Sequence: Synthetic primer"
gccgtaggtggtcacgagggtgg

SEQ ID NO: 110 - DNA, 23 bp, Artificial Sequence
  source: /note="Description of Artificial Sequence: Synthetic primer"
gcacgccgtaggtggtcacgagg

SEQ ID NO: 111 - DNA, 23 bp, Artificial Sequence
  source: /note="Description of Artificial Sequence: Synthetic primer"
cccaccctcgtgaccacctacgg

SEQ ID NO: 112 - DNA, 23 bp, Artificial Sequence
  source: /note="Description of Artificial Sequence: Synthetic primer"
gaagcactgcacgccgtaggtgg

SEQ ID NO: 113 - DNA, 23 bp, Artificial Sequence
  source: /note="Description of Artificial Sequence: Synthetic primer"
ggcgaagcactgcacgccgtagg

SEQ ID NO: 114 - DNA, 23 bp, Artificial Sequence
  source: /note="Description of Artificial Sequence: Synthetic primer"
cttcatgtggtcggggtagcggg

SEQ ID NO: 115 - DNA, 23 bp, Artificial Sequence
  source: /note="Description of Artificial Sequence: Synthetic primer"
gtcgtgctgcttcatgtggtcgg

SEQ ID NO: 116 - DNA, 23 bp, Artificial Sequence
  source: /note="Description of Artificial Sequence: Synthetic primer"
agaagtcgtgctgcttcatgtgg

SEQ ID NO: 117 - DNA, 23 bp, Artificial Sequence
  source: /note="Description of Artificial Sequence: Synthetic primer"
gcatttctcagtcctaaacaggg

SEQ ID NO: 118 - DNA, 20 bp, Artificial Sequence
  source: /note="Description of Artificial Sequence: Synthetic primer"
agcggctctagtatcaaccc

SEQ ID NO: 119 - DNA, 20 bp, Artificial Sequence
  source: /note="Description of Artificial Sequence: Synthetic primer"
aagatatgtagccgccctac

SEQ ID NO: 120 - DNA, 20 bp, Artificial Sequence
  source: /note="Description of Artificial Sequence: Synthetic primer"
ccggtcaatgagcactattt

SEQ ID NO: 121 - DNA, 720 bp, Artificial Sequence
  source: /note="Description of Artificial Sequence: Synthetic polynucleotide"
atggtgagcaagggcgaggagctgttcaccggggtggtgcccatcctggtcgagctggacggcgacgtaaacggccacaagttcagcgtgtccggcgagggcgagggcgatgccacctacggcaagctgaccctgaagttcatctgcaccaccggcaagctgcccgtgccctggcccaccctcgtgaccaccttcacctacggcgtgcagtgcttcgcccgctaccccgaccacatgaagcagcacgacttcttcaagtccgccatgcccgaaggctacgtccaggagcgcaccatcttcttcaaggacgacggcaactacaagacccgcgccgaggtgaagttcgagggcgacaccctggtgaaccgcatcgagctgaagggcatcgacttcaaggaggacggcaacatcctggggcacaagctggagtacaactacaacagccacaaggtctatatcaccgccgacaagcagaagaacggcatcaaggtgaacttcaagacccgccacaacatcgaggacggcagcgtgcagctcgccgaccactaccagcagaacacccccatcggcgacggccccgtgctgctgcccgacaaccactacctgagcacccagtccgccctgagcaaagaccccaacgagaagcgcgatcacatggtcctgctggagttcgtgaccgccgccgggatcactctcggcatggacgagctgtacaagtaa

SEQ ID NO: 122 - DNA, 714 bp, Artificial Sequence
  source: /note="Description of Artificial Sequence: Synthetic polynucleotide"
atggtgagcaagggcgaggagctgttcaccggggtggtgcccatcctggtcgagctggacggcgacgtaaacggccacaagttcagcgtgtccggcgagggcgagggcgatgccacctacggcaagctgaccctgaagttcatctgcaccaccggcaagctgcccgtgccctggcccaccctcgtgaccacctacggcgtgcagtgcttcgcccgctaccccgaccacatgaagcagcacgacttcttcaagtccgccatgcccgaaggctacgtccaggagcgcaccatcttcttcaaggacgacggcaactacaagacccgcgccgaggtgaagttcgagggcgacaccctggtgaaccgcatcgagctgaagggcatcgacttcaaggaggacggcaacatcctggggcacaagctggagtacaactacaacagccacaaggtctatatcaccgccgacaagcagaagaacggcatcaaggtgaacttcaagacccgccacaacatcgaggacggcagcgtgcagctcgccgaccactaccagcagaacacccccatcggcgacggccccgtgctgctgcccgacaaccactacctgagcacccagtccgccctgagcaaagaccccaacgagaagcgcgatcacatggtcctgctggagttcgtgaccgccgccgggatcactctcggcatggacgagctgtacaagtaa

SEQ ID NO: 123 - DNA, 720 bp, Artificial Sequence
  source: /note="Description of Artificial Sequence: Synthetic polynucleotide"
atggtgagcaagggcgaggagctgttcaccggggtggtgcccatcctggtcgagctggacggcgacgtaaacggccacaagttcagcgtgtccggcgagggcgagggcgatgccacctacggcaagctgaccctgaagttcatctgcaccaccggcaagctgcccgtgccctggcccaccctcgtgaccaccctgacccacggcgtgcagtgcttcagccgctaccccgaccacatgaagcagcacgacttcttcaagtccgccatgcccgaaggctacgtccaggagcgcaccatcttcttcaaggacgacggcaactacaagacccgcgccgaggtgaagttcgagggcgacaccctggtgaaccgcatcgagctgaagggcatcgacttcaaggaggacggcaacatcctggggcacaagctggagtacaactacaacagccacaacgtctatatcatggccgacaagcagaagaacggcatcaaggtgaacttcaagatccgccacaacatcgaggacggcagcgtgcagctcgccgaccactaccagcagaacacccccatcggcgacggccccgtgctgctgcccgacaaccactacctgagcacccagtccgccctgagcaaagaccccaacgagaagcgcgatcacatggtcctgctggagttcgtgaccgccgccgggatcactctcggcatggacgagctgtacaagtaa

SEQ ID NO: 124 - DNA, 720 bp, Artificial Sequence
  source: /note="Description of Artificial Sequence: Synthetic polynucleotide"
atggtgagcaagggcgaggagctgttcaccggggtggtgcccatcctggtcgagctggacggcgacgtaaacggccacaagttcagcgtgtccggcgagggcgagggcgatgccacctacggcaagctgaccctgaagttcatctgcaccaccggcaagctgcccgtgccctggcccaccctcgtgaccaccctgacctacggcgtgcagtgcttcagccgctaccccgaccacatgaagcagcacgacttcttcaagtccgccatgcccgaaggctacgtccaggagcgcaccatcttcttcaaggacgacggcaactacaagacccgcgccgaggtgaagttcgagggcgacaccctggtgaaccgcatcgagctgaagggcatcgacttcaaggaggacggcaacatcctggggcacaagctggagtacaactacaacagccacaacgtctatatcatggccgacaagcagaagaacggcatcaaggtgaacttcaagatccgccacaacatcgaggacggcagcgtgcagctcgccgaccactaccagcagaacacccccatcggcgacggccccgtgctgctgcccgacaaccactacctgagcacccagtccgccctgagcaaagaccccaacgagaagcgcgatcacatggtcctgctggagttcgtgaccgccgccgggatcactctcggcatggacgagctgtacaagtaa

SEQ ID NO: 125 - DNA, 23 bp, Artificial Sequence
  source: /note="Description of Artificial Sequence: Synthetic oligonucleotide"
ctcgtgaccaccttcacctacgg

SEQ ID NO: 126 - DNA, 24 bp, Artificial Sequence
  source: /note="Description of Artificial Sequence: Synthetic primer"
atggtgagcaagggcgaggagctg

SEQ ID NO: 127 - DNA, 22 bp, Artificial Sequence
  source: /note="Description of Artificial Sequence: Synthetic primer"
gtcctccttgaagtcgatgccc